European Patent Application EP 4 450 623 A1, published October 23, 2024. Title: miRNA-2911分子作为核酸稳定剂的应用. Applicant: 成都凌泰氪生物技术有限公司. Application CN. The sequence listing filed with the application follows.

SEQUENCE LISTING (29 sequences)

SEQ ID NO: 1 - RNA, 21 nt, synthetic construct
  source 1..21: mol_type = other RNA
  misc_feature 3..4: note = a c t u
  misc_feature 10: note = a c t u; number = 10
  misc_feature 15..17: note = a c t u
  misc_feature 11..12: note = a c t u
  misc_feature 21: note = a c t u
ggnngggggnnnggnnngggn

SEQ ID NO: 2 - RNA, 20 nt, synthetic construct
  source 1..20: mol_type = other RNA
ggccgggggacggactggga

SEQ ID NO: 3 - RNA, 20 nt, synthetic construct
  source 1..20: mol_type = other RNA
  misc_feature 3..4: note = a c t u
  misc_feature 10..11: note = a c t u
  misc_feature 14..16: note = a c t u
  misc_feature 20: note = a c t u
ggnngggggnnggnnngggn

SEQ ID NO: 4 - RNA, 20 nt, synthetic construct
  source 1..20: mol_type = other RNA
ggaagggggaaggaaaggga

SEQ ID NO: 5 - RNA, 20 nt, synthetic construct
  source 1..20: mol_type = other RNA
ggccgggggccggcccgggc

SEQ ID NO: 6 - RNA, 20 nt, synthetic construct
  source 1..20: mol_type = other RNA
ggttgggggttggtttgggt

SEQ ID NO: 7 - RNA, 25 nt, synthetic construct
  source 1..25: mol_type = other RNA
ggaaggggggggggaaggaaaggga

SEQ ID NO: 8 - RNA, 40 nt, synthetic construct
  source 1..40: mol_type = other RNA
ggaagggggaaggaaagggaggaagggggaaggaaaggga

SEQ ID NO: 9 - DNA, 20 bp, synthetic construct
  source 1..20: mol_type = other DNA
ggccgggggacggactggga

SEQ ID NO: 10 - DNA, 20 bp, synthetic construct
  source 1..20: mol_type = other DNA
ggaagggggaaggaaaggga

SEQ ID NO: 11 - RNA, 20 nt, synthetic construct
  source 1..20: mol_type = other RNA
tgaatgtagagatgcggtgg

SEQ ID NO: 12 - RNA, 59 nt, synthetic construct
  source 1..59: mol_type = other RNA
acccgacctcttctatctggacccgaccgtctcttttttgagcccacactctactcgac

SEQ ID NO: 13 - DNA, 20 bp, synthetic construct
  source 1..20: mol_type = other DNA
tgaatgtagagatgcggtgg

SEQ ID NO: 14 - DNA, 60 bp, synthetic construct
  source 1..60: mol_type = other DNA
  misc_feature 1..20: note = RNA
  misc_feature 41..60: note = RNA
tgaatgtagagatgcggtggtgaatgtagagatgcggtggtgaatgtagagatgcggtgg

SEQ ID NO: 15 - DNA, 60 bp, synthetic construct
  source 1..60: mol_type = other DNA
  misc_feature 21..40: note = RNA
ggaagggggaaggaaagggatgaatgtagagatgcggtggggaagggggaaggaaaggga

SEQ ID NO: 16 - DNA, 60 bp, synthetic construct
  source 1..60: mol_type = other DNA
atttgacctcttctatctggacccgaccgtctcttttttgagcccacactctactcgacg

SEQ ID NO: 17 - RNA, 20 nt, synthetic construct
  source 1..20: mol_type = other RNA
acggggtcattagttcatag

SEQ ID NO: 18 - RNA, 20 nt, synthetic construct
  source 1..20: mol_type = other RNA
taagatacacctgcaaaggc

SEQ ID NO: 19 - RNA, 20 nt, synthetic construct
  source 1..20: mol_type = other RNA
gctctcctcaagcgtattca

SEQ ID NO: 20 - RNA, 20 nt, synthetic construct
  source 1..20: mol_type = other RNA
gtcgagctggacggcgacgt

SEQ ID NO: 21 - RNA, 20 nt, synthetic construct
  source 1..20: mol_type = other RNA
tgaccctgaagttcatctgc

SEQ ID NO: 22 - RNA, 120 nt, synthetic construct
  source 1..120: mol_type = other RNA
ggaagggggaaggaaagggagctgtgtgactcctgcaaagtgtggacaacttcccacggaggaattcccgtatctaaaggtgcagctgtatcttgtctccggaagggggaaggaaaggga

SEQ ID NO: 23 - RNA, 80 nt, synthetic construct
  source 1..80: mol_type = other RNA
aacctcttagacaggtgggagattatgatcagagtaaaaggtaattacacattttatttccagaaagtcaggggtctata

SEQ ID NO: 24 - RNA, 2040 nt, synthetic construct
  source 1..2040: mol_type = other RNA
ggaagggggaaggaaagggattatttttaagagctgtggagttcttaaatatcaaccatggcactttctcctgaccccttccctaggggatttcaggattgagaaatttttccatcgagcctttttaaaattgtaggacttgttcctgtgggcttcagtgatgggatagtacacttcactcagaggcatttgcatctttaaataatttcttaaaagcctctaaagtgatcagtgccttgatgccaactaaggaaatttgtttagcattgaatctctgaaggctctatgaaaggaatagcatgatgtgctgttagaatcagatgttactgctaaaatttacatgttgtgatgtaaattgtgtagaaaaccattaaatcattcaaaataataaactatttttattagagaatgtatacttttagaaagctgtctccttatttaaataaaatagtgtttgtctgtagttcagtgttggggcaatcttgggggggattcttctctaatctttcagaaactttgtctgcgaacactctttaatggaccagatcaggatttgagcggaagaacgaatgtaactttaaggcaggaaagacaaattttattcttcataaagtgatgagcatataataattccaggcacatggcaatagaggccctctaaataaggaataaataacctcttagacaggtgggagattatgatcagagtaaaaggtaattacacattttatttccagaaagtcaggggtctataaattgacagtgattagagtaatactttttcacatttccaaagtttgcatgttaactttaaatgcttacaatcttagagtggtaggcaatgttttacactattgaccttatatagggaagggagggggtgcctgtggggttttaaagaattttcctttgcagaggcatttcatccttcatgaagccattcaggattttgaattgcatatgagtgcttggctcttccttctgttctagtgagtgtatgagaccttgcagtgagtttatcagcatactcaaaatttttttcctggaatttggagggatgggaggagggggtggggcttacttgttgtagctttttttttttttacagacttcacagagaatgcagttgtcttgacttcaggtctgtctgttctgttggcaagtaaatgcagtactgttctgatcccgctgctattagaatgcattgtgaaacgactggagtatgattaaaagttgtgttccccaatgcttggagtagtgattgttgaaggaaaaaatccagctgagtgataaaggctgagtgttgaggaaatttctgcagttttaagcagtcgtatttgtgattgaagctgagtacattttgctggtgtatttttaggtaaaatgctttttgttcatttctggtggtgggaggggactgaagcctttagtcttttccagatgcaaccttaaaatcagtgacaagaaacattccaaacaagcaacagtcttcaagaaattaaactggcaagtggaaatgtttaaacagttcagtgatctttagtgcattgtttatgtgtgggtttctctctcccctcccttggtcttaattcttacatgcaggaacactcagcagacacacgtatgcgaagggccagagaagccagacccagtaagaaaaaatagcctatttactttaaataaaccaaacattccattttaaatgtggggattgggaaccactagttctttcagatggtattcttcagactatagaaggagcttccagttgaattcaccagtggacaaaatgaggaaaacaggtgaacaagctttttctgtatttacatacaaagtcagatcagttatgggacaatagtattgaatagatttcagctttatgctggagtaactggcatgtgagcaaactgtgttggcgtgggggtggaggggtgaggtgggcgctaagcctttttttaagatttttcaggtacccctcactaaaggcaccgaaggcttaaagtaggacaaccatggagccggaagggggaaggaaaggga

SEQ ID NO: 25 - RNA, 2000 nt, synthetic construct
  source 1..2000: mol_type = other RNA
ttatttttaagagctgtggagttcttaaatatcaaccatggcactttctcctgaccccttccctaggggatttcaggattgagaaatttttccatcgagcctttttaaaattgtaggacttgttcctgtgggcttcagtgatgggatagtacacttcactcagaggcatttgcatctttaaataatttcttaaaagcctctaaagtgatcagtgccttgatgccaactaaggaaatttgtttagcattgaatctctgaaggctctatgaaaggaatagcatgatgtgctgttagaatcagatgttactgctaaaatttacatgttgtgatgtaaattgtgtagaaaaccattaaatcattcaaaataataaactatttttattagagaatgtatacttttagaaagctgtctccttatttaaataaaatagtgtttgtctgtagttcagtgttggggcaatcttgggggggattcttctctaatctttcagaaactttgtctgcgaacactctttaatggaccagatcaggatttgagcggaagaacgaatgtaactttaaggcaggaaagacaaattttattcttcataaagtgatgagcatataataattccaggcacatggcaatagaggccctctaaataaggaataaataacctcttagacaggtgggagattatgatcagagtaaaaggtaattacacattttatttccagaaagtcaggggtctataaattgacagtgattagagtaatactttttcacatttccaaagtttgcatgttaactttaaatgcttacaatcttagagtggtaggcaatgttttacactattgaccttatatagggaagggagggggtgcctgtggggttttaaagaattttcctttgcagaggcatttcatccttcatgaagccattcaggattttgaattgcatatgagtgcttggctcttccttctgttctagtgagtgtatgagaccttgcagtgagtttatcagcatactcaaaatttttttcctggaatttggagggatgggaggagggggtggggcttacttgttgtagctttttttttttttacagacttcacagagaatgcagttgtcttgacttcaggtctgtctgttctgttggcaagtaaatgcagtactgttctgatcccgctgctattagaatgcattgtgaaacgactggagtatgattaaaagttgtgttccccaatgcttggagtagtgattgttgaaggaaaaaatccagctgagtgataaaggctgagtgttgaggaaatttctgcagttttaagcagtcgtatttgtgattgaagctgagtacattttgctggtgtatttttaggtaaaatgctttttgttcatttctggtggtgggaggggactgaagcctttagtcttttccagatgcaaccttaaaatcagtgacaagaaacattccaaacaagcaacagtcttcaagaaattaaactggcaagtggaaatgtttaaacagttcagtgatctttagtgcattgtttatgtgtgggtttctctctcccctcccttggtcttaattcttacatgcaggaacactcagcagacacacgtatgcgaagggccagagaagccagacccagtaagaaaaaatagcctatttactttaaataaaccaaacattccattttaaatgtggggattgggaaccactagttctttcagatggtattcttcagactatagaaggagcttccagttgaattcaccagtggacaaaatgaggaaaacaggtgaacaagctttttctgtatttacatacaaagtcagatcagttatgggacaatagtattgaatagatttcagctttatgctggagtaactggcatgtgagcaaactgtgttggcgtgggggtggaggggtgaggtgggcgctaagcctttttttaagatttttcaggtacccctcactaaaggcaccgaaggcttaaagtaggacaaccatggagcc

SEQ ID NO: 26 - RNA, 60 nt, synthetic construct
  source 1..60: mol_type = other RNA
tgaatgtagagatgcggtggggaagggggaaggaaagggatgaatgtagagatgcggtgg

SEQ ID NO: 27 - RNA, 40 nt, synthetic construct
  source 1..40: mol_type = other RNA
ggaagggggaaggaaagggatgaatgtagagatgcggtgg

SEQ ID NO: 28 - RNA, 40 nt, synthetic construct
  source 1..40: mol_type = other RNA
tgaatgtagagatgcggtggggaagggggaaggaaaggga

SEQ ID NO: 29 - RNA, 40 nt, synthetic construct
  source 1..40: mol_type = other RNA
acccgacctcttctatctggacccgaccgtctcttttttg